European Patent Application EP 4 596 576 A1, published August 6, 2025. Title: 신규한 재조합 Fc 수용체 및 이를 포함하는 세포. Applicant: 카오티에스. Application KR. The sequence listing filed with the application follows.

SEQUENCE LISTING (9 sequences)

SEQ ID NO: 1 - protein, 254 aa, synthetic construct
MWQLLLPTALLLLVSAGMRTEDLPKAVVFLEPQWYRVLEKDSVTLKCQGAYSPEDNSTQWFHNESLISSQASSYFIDAATVDDSGEYRCQTNLSTLSDPVQLEVHIGWLLLQAPRWVFKEEDPIHLRCHSWKNTALHKVTYLQNGKGRKYFHHNSDFYIPKATLKDSGSYFCRGLFGSKNVSSETVNITITQGLAVSTISSFFPPGYQVSFCLVMVLLFAVDTGLYFSVKTNIRSSTRDWKDHKFKWRKDPQDK

SEQ ID NO: 2 - protein, 283 aa, synthetic construct
MWFLTTLLLWVPVDGQVDTTKAVITLQPPWVSVFQEETVTLHCEVLHLPGSSSTQWFLNGTATQTSTPSYRITSASVNDSGEYRCQRGLSGRSDPIQLEIHRGWLLLQVSSRVFTEGEPLALRCHAWKDKLVYNVLYYRNGKAFKFFHWNSNLTILKTNISHNGTYHCSGMGKHRYTSAGISVTVKELFPAPVLNASVTSPLLEGNLVTLSCETKLLLQRPGLQLYFSFYMGSKTLRGRNTSSEYQILTARREDSGLYWCEAATEDGNVLKRSPELELQVLGL

SEQ ID NO: 3 - protein, 280 aa, synthetic construct
MWFLTTLLLWVPVDGQVDTTKAVITLQPPWVSVFQEETVTLHCEVLHLPGSSSTQWFLNGTATQTSTPSYRITSASVNDSGEYRCQRGLSGRSDPIQLEIHRGWLLLQVSSRVFTEGEPLALRCHAWKDKLVYNVLYYRNGKAFKFFHWNSNLTILKTNISHNGTYHCSGMGKHRYTSAGISVTVKELFPAPVLNASVTSPLLEGNLVTLSCETKLLLQRPGLQLYFSFYMGSKTLRGRNTSSEYQILTARREDSGLYWCEAATEDGNVLKRSPELELQV

SEQ ID NO: 4 - protein, 254 aa, synthetic construct
MWQLLLPTALLLLVSAGMRTEDLPKAVVFLEPQWYRVLEKDSVTLKCQGAYSPEDNSTQWFHNESLISSQASSYFIDAATVDDSGEYRCQTNLSTLSDPVQLEVHIGWLLLQAPRWVFKEEDPIHLRCHSWKNTALHKVTYLQNGKGRKYFHHNSDFYIPKATLKDSGSYFCRGLVGSKNVSSETVNITITQGLAVPSISSFFPPGYQVSFCLVMVLLFAVDTGLYFSVKTNIRSSTRDWKDHKFKWRKDPQDK

SEQ ID NO: 5 - protein, 343 aa, synthetic construct
MWFLTTLLLWVPVDGQVDTTKAVITLQPPWVSVFQEETVTLHCEVLHLPGSSSTQWFLNGTATQTSTPSYRITSASVNDSGEYRCQRGLSGRSDPIQLEIHRGWLLLQVSSRVFTEGEPLALRCHAWKDKLVYNVLYYRNGKAFKFFHWNSNLTILKTNISHNGTYHCSGMGKHRYTSAGISVTVKELFPAPVLNASVTSPLLEGNLVTLSCETKLLLQRPGLQLYFSFYMGSKTLRGRNTSSEYQILTARREDSGLYWCEAATEDGNVLKRSPELELQVLGLAVPTISSFFPPGYQVSFCLVMVLLFAVDTGLYFSVKTNIRSSTRDWKDHKFKWRKDPQDK

SEQ ID NO: 6 - protein, 343 aa, synthetic construct
MWFLTTLLLWVPVDGQVDTTKAVITLQPPWVSVFQEETVTLHCEVLHLPGSSSTQWFLNGTATQTSTPSYRITSASVNDSGEYRCQRGLSGRSDPIQLEIHRGWLLLQVSSRVFTEGEPLALRCHAWKDKLVYNVLYYRNGKAFKFFHWNSNLTILKTNISHNGTYHCSGMGKHRYTSAGISVTVKELFPAPVLNASVTSPLLEGNLVTLSCETKLLLQRPGLQLYFSFYMGSKTLRGRNTSSEYQILTARREDSGLYWCEAATEDGNVLKRSPELELQVLGLAVPSISSFFPPGYQVSFCLVMVLLFAVDTGLYFSVKTNIRSSTRDWKDHKFKWRKDPQDK

SEQ ID NO: 7 - protein, 343 aa, synthetic construct
MWFLTTLLLWVPVDGQVDTTKAVITLQPPWVSVFQEETVTLHCEVLHLPGSSSTQWFLNGTATQTSTPSYRITSASVNDSGEYRCQRGLSGRSDPIQLEIHRGWLLLQVSSRVFTEGEPLALRCHAWKDKLVYNVLYYRNGKAFKFFHWNSNLTILKTNISHNGTYHCSGMGKHRYTSAGISVTVKELFPAPVLNASVTSPLLEGNLVTLSCETKLLLQRPGLQLYFSFYMGSKTLRGRNTSSEYQILTARREDSGLYWCEAATEDGNVLKRSPELELQVQGLAVPSISSFFPPGYQVSFCLVMVLLFAVDTGLYFSVKTNIRSSTRDWKDHKFKWRKDPQDK

SEQ ID NO: 8 - protein, 343 aa, synthetic construct
MWFLTTLLLWVPVDGQVDTTKAVITLQPPWVSVFQEETVTLHCEVLHLPGSSSTQWFLNGTATQTSTPSYRITSASVNDSGEYRCQRGLSGRSDPIQLEIHRGWLLLQVSSRVFTEGEPLALRCHAWKDKLVYNVLYYRNGKAFKFFHWNSNLTILKTNISHNGTYHCSGMGKHRYTSAGISVTVKELFPAPVLNASVTSPLLEGNLVTLSCETKLLLQRPGLQLYFSFYMGSKTLRGRNTSSEYQILTARREDSGLYWCEAATEDGNVLKRSPELELQVLGLAVSTISSFFPPGYQVSFCLVMVLLFAVDTGLYFSVKTNIRSSTRDWKDHKFKWRKDPQDK

SEQ ID NO: 9 - protein, 254 aa, synthetic construct
MWQLLLPTALLLLVSAGMRTEDLPKAVVFLEPQWYRVLEKDSVTLKCQGAYSPEDNSTQWFHNESLISSQASSYFIDAATVDDSGEYRCQTNLSTLSDPVQLEVHIGWLLLQAPRWVFKEEDPIHLRCHSWKNTALHKVTYLQNGKGRKYFHHNSDFYIPKATLKDSGSYFCRGLVGSKNVSSETVNITITQGLAVSTISSFFPPGYQVSFCLVMVLLFAVDTGLYFSVKTNIRSSTRDWKDHKFKWRKDPQDK